European Patent Specification EP 4 059 953 B1, published October 23, 2024. Title: Novel protein variant and a method for producing L-valine using the same. Applicant: CJ CheilJedang Corporation. The sequence listing filed with the application follows.

SEQUENCE LISTING (11 sequences)

SEQ ID NO: 1 - protein, 297 aa, Artificial Sequence
  Protein variant
MLDTFHLSVLSEDEWMELARAHHARADSFTKDHLKRRQAHIKHPVFDFLFEYYPVRVAHLKTWHPGIGVFLEGTPPHATMRDFLLVDASLHHAAGVQLDLASYMQRRGFSVRYIHELLSATRDNHAQFDCFGLHEWAMVYKSNDLRHDLPLRLTPSETDRVVESHNIKCTHFDAYRFFTTPAIPLNLTVLTREDQPRNDQCGCLHATMDLYKWSAKLGPLVPGDLFLEAFELARDTRILDMEASPYDVRGYGFGYVPIETAEGKAEYVSRQRELSERAKPIRDRLVSITKQALQASI

SEQ ID NO: 2 - DNA, 894 bp, Artificial Sequence
  Protein variant coding gene
gtgttggacacttttcacctcagcgtattgagcgaggatgagtggatggaactagcccgcgcccaccacgcgcgggctgattcattcaccaaagaccacttgaagcgtcgacaagcgcatatcaagcaccccgtcttcgacttcctcttcgagtactaccccgtgcgcgtcgcgcacctaaaaacctggcaccccggcatcggcgtgttcctagaaggcacaccgccgcatgccaccatgcgcgattttttgcttgtcgacgcctccctccatcacgcagctggcgtccagcttgacctggcctcctatatgcaacgccgtgggttctctgtgcgctacatccacgaactgttgtccgccacccgtgacaaccacgcccaatttgattgttttggtctgcacgaatgggcaatggtgtacaaatcaaacgatctccgccatgatcttcccctgcgccttaccccatcggaaaccgaccgtgtggtggaaagccacaacatcaaatgcacccactttgatgcctaccgattcttcaccacaccagccatcccgttgaacctcacggtgttaacccgcgaagatcagccacgcaacgatcaatgcggttgtctgcatgccacgatggatctatacaaatggtccgcaaagcttggccctcttgtgccaggtgatcttttcttggaagcgtttgaactagcccgcgacacccgcatcttggacatggaggcttcgccttacgacgtccgcggatacggctttggctacgtccccattgagaccgccgagggcaaagccgaatatgtcagtagacaacgcgagctgtctgaacgagcaaaacccatccgtgaccggcttgtctccattactaaacaagctctacaggctagtatttag

SEQ ID NO: 3 - protein, 297 aa, Artificial Sequence
  Wild type protein
MLDTFHLSVLSEDEWMELARAHHARADSFTKDHLKRRQAHIKHPVFDFLFEYYPVRVAHLKTWHPGIGVFLEGTPPHATMRDFLLVDASLHHAAGVQLDLASYMQRRGSSVRYIHELLSATRDNHAQFDCFGLHEWAMVYKSNDLRHDLPLRLTPSETDRVVESHNIKCTHFDAYRFFTTPAIPLNLTVLTREDQPRNDQCGCLHATMDLYKWSAKLGPLVPGDLFLEAFELARDTRILDMEASPYDVRGYGFGYVPIETAEGKAEYVSRQRELSERAKPIRDRLVSITKQALQASI

SEQ ID NO: 4 - DNA, 894 bp, Artificial Sequence
  Wild type protein coding gene
gtgttggacacttttcacctcagcgtattgagcgaggatgagtggatggaactagcccgcgcccaccacgcgcgggctgattcattcaccaaagaccacttgaagcgtcgacaagcgcatatcaagcaccccgtcttcgacttcctcttcgagtactaccccgtgcgcgtcgcgcacctaaaaacctggcaccccggcatcggcgtgttcctagaaggcacaccgccgcatgccaccatgcgcgattttttgcttgtcgacgcctccctccatcacgcagctggcgtccagcttgacctggcctcctatatgcaacgccgtgggtcctctgtgcgctacatccacgaactgttgtccgccacccgtgacaaccacgcccaatttgattgttttggtctgcacgaatgggcaatggtgtacaaatcaaacgatctccgccatgatcttcccctgcgccttaccccatcggaaaccgaccgtgtggtggaaagccacaacatcaaatgcacccactttgatgcctaccgattcttcaccacaccagccatcccgttgaacctcacggtgttaacccgcgaagatcagccacgcaacgatcaatgcggttgtctgcatgccacgatggatctatacaaatggtccgcaaagcttggccctcttgtgccaggtgatcttttcttggaagcgtttgaactagcccgcgacacccgcatcttggacatggaggcttcgccttacgacgtccgcggatacggctttggctacgtccccattgagaccgccgagggcaaagccgaatatgtcagtagacaacgcgagctgtctgaacgagcaaaacccatccgtgaccggcttgtctccattactaaacaagctctacaggctagtatttag

SEQ ID NO: 5 - DNA, 36 bp, Artificial Sequence
  NCgl1391_1F
tcgagctcggtacccacggcctcatggatgacgtct

SEQ ID NO: 6 - DNA, 44 bp, Artificial Sequence
  NCgl1391_2R
tcgtggatgtagcgcacagagaacccacggcgttgcatatagga

SEQ ID NO: 7 - DNA, 44 bp, Artificial Sequence
  NCgl1391_3F
tcctatatgcaacgccgtgggttctctgtgcgctacatccacga

SEQ ID NO: 8 - DNA, 36 bp, Artificial Sequence
  NCgl1391_4R
ctctagaggatcccctttgctcgttcagacagctcg

SEQ ID NO: 9 - DNA, 21 bp, Artificial Sequence
  NCgl1391_5F
acggcctcatggatgacgtct

SEQ ID NO: 10 - DNA, 21 bp, Artificial Sequence
  NCgl1391_6R
tttgctcgttcagacagctcg

SEQ ID NO: 11 - DNA, 5803 bp, Artificial Sequence
  pDCM2
gttcgcttgctgtccataaaaccgcccagtctagctatcgccatgtaagcccactgcaagctacctgctttctctttgcgcttgcgttttcccttgtccagatagcccagtagctgacattcatccggggtcagcaccgtttctgcggactggctttctacgtgttccgcttcctttagcagcccttgcgccctgagtgcttgcggcagcgtgaagctagcttttatcgccattcgccattcaggctgcgcaactgttgggaagggcgatcggtgcgggcctcttcgctattacgccagctggcgaaagggggatgtgctgcaaggcgattaagttgggtaacgccagggttttcccagtcacgacgttgtaaaacgacggccagtgaattcgagctcggtacccggggatcctctagagtcgacctgcaggcatgcaagcttggcgtaatcatggtcatagctgtttcctgtgtgaaattgttatccgctcacaattccacacaacatacgagccggaagcataaagtgtaaagcctggggtgcctaatgagtgagctaactcacattaattgcgttgcgctcactgcccgctttccagtcgggaaacctgtcgtgccagctgcattaatgaatcggccaacgcgcggggagaggcggtttgcgtattgggcgctcttccgcttcctcgctcactgactcgctgcgctcggtcgttcggctgcggcgagcggtatcagctcactcaaaggcggtaatacggttatccacagaatcaggggataacgcaggaaagaacatgtgagcaaaaggccagcaaaaggccaggaaccgtaaaaaggccgcgttgctggcgtttttccataggctccgcccccctgacgagcatcacaaaaatcgacgctcaagtcagaggtggcgaaacccgacaggactataaagataccaggcgtttccccctggaagctccctcgtgcgctctcctgttccgaccctgccgcttaccggatacctgtccgcctttctcccttcgggaagcgtggcgctttctcaatgctcacgctgtaggtatctcagttcggtgtaggtcgttcgctccaagctgggctgtgtgcacgaaccccccgttcagcccgaccgctgcgccttatccggtaactatcgtcttgagtccaacccggtaagacacgacttatcgccactggcagcagccactggtaacaggattagcagagcgaggtatgtaggcggtgctacagagttcttgaagtggtggcctaactacggctacactagaaggacagtatttggtatctgcgctctgctgaagccagttaccttcggaaaaagagttggtagctcttgatccggcaaacaaaccaccgctggtagcggtggtttttttgtttgcaagcagcagattacgcgcagaaaaaaaggatctcaagaagatcctttgatcttttctacggggtctgacgctcagtggaacgaaaactcacgttaagggattttggtcatgagattatcaaaaaggatcttcacctagatccttttggggtgggcgaagaactccagcatgagatccccgcgctggaggatcatccagccctgatagaaacagaagccactggagcacctcaaaaacaccatcatacactaaatcagtaagttggcagcatcacccgacgcactttgcgccgaataaatacctgtgacggaagatcacttcgcagaataaataaatcctggtgtccctgttgataccgggaagccctgggccaacttttggcgaaaatgagacgttgatcggcacgtaagaggttccaactttcaccataatgaaataagatcactaccgggcgtattttttgagttatcgagattttcaggagctgatagaaacagaagccactggagcacctcaaaaacaccatcatacactaaatcagtaagttggcagcatcacccgacgcactttgcgccgaataaatacctgtgacggaagatcacttcgcagaataaataaatcctggtgtccctgttgataccgggaagccctgggccaacttttggcgaaaatgagacgttgatcggcacgtaagaggttccaactttcaccataatgaaataagatcactaccgggcgtattttttgagttatcgagattttcaggagctctttggcatcgtctctcgcctgtcccctcagttcagtaatttcctgcatttgcctgtttccagtcggtagatattccacaaaacagcagggaagcagcgcttttccgctgcataaccctgcttcggggtcattatagcgattttttcggtatatccatcctttttcgcacgatatacaggattttgccaaagggttcgtgtagactttccttggtgtatccaacggcgtcagccgggcaggataggtgaagtaggcccacccgcgagcgggtgttccttcttcactgtcccttattcgcacctggcggtgctcaacgggaatcctgctctgcgaggctggccggctaccgccggcgtaacagatgagggcaagcggatggctgatgaaaccaagccaaccaggaagggcagcccacctatcaaggtgtactgccttccagacgaacgaagagcgattgaggaaaaggcggcggcggccggcatgagcctgtcggcctacctgctggccgtcggccagggctacaaaatcacgggcgtcgtggactatgagcacgtccgcgagggcgtcccggaaaacgattccgaagcccaacctttcatagaaggcggcggtggaatcgaaatctcgtgatggcaggttgggcgtcgcttggtcggtcatttcgaaaaaggttaggaatacggttagccatttgcctgcttttatatagttcantatgggattcacctttatgttgataagaaataaaagaaaatgccaataggatatcggcattttcttttgcgtttttatttgttaactgttaattgtccttgttcaaggatgctgtctttgacaacagatgttttcttgcctttgatgttcagcaggaagctcggcgcaaacgttgattgtttgtctgcgtagaatcctctgtttgtcatatagcttgtaatcacgacattgtttcctttcgcttgaggtacagcgaagtgtgagtaagtaaaggttacatcgttaggcggatcaagatccatttttaacacaaggccagttttgttcagcggcttgtatgggccagttaaagaattagaaacataaccaagcatgtaaatatcgttagacgtaatgccgtcaatcgtcatttttgatccgcgggagtcagtgaacaggtaccatttgccgttcattttaaagacgttcgcgcgttcaatttcatctgttactgtgttagatgcaatcagcggtttcatcacttttttcagtgtgtaatcatcgtttagctcaatcataccgagagcgccgtttgctaactcagccgtgcgttttttatcgctttgcagaagtttttgactttcttgacggaagaatgatgtgcttttgccatagtatgctttgttaaataaagattcttcgccttggtagccatcttcagttccagtgtttgcttcaaatactaagtatttgtggcctttatcttctacgtagtgaggatctctcagcgtatggttgtcgcctgagctgtagttgccttcatcgatgaactgctgtacattttgatacgtttttccgtcaccgtcaaagattgatttataatcctctacaccgttgatgttcaaagagctgtctgatgctgatacgttaacttgtgcagttgtcagtgtttgtttgccgtaatgtttaccggagaaatcagtgtagaataaacggatttttccgtcagatgtaaatgtggctgaacctgaccattcttgtgtttggtcttttaggatagaatcatttgcatcgaatttgtcgctgtctttaaagacgcggccagcgtttttccagctgtcaatagaagtttcgccgactttttgatagaacatgtaaatcgatgtgtcatccgcatttttaggatctccggctaatgcaaagacgatgtggtagccgtgatagtttgcgacagtgccgtcagcgttttgtaatggccagctgtcccaaacgtccaggccttttgcagaagagatatttttaattgtggacgaatcaaattcagaaacttgatatttttcatttttttgctgttcagggatttgcagcatatcatggcgtgtaatatgggaaatgccgtatgtttccttatatggcttttggttcgtttctttcgcaaacgcttgagttgcgcctcctgccagcagtgcggtagtaaaggttaatactgttgcttgttttgcaaactttttgatgttcatcgttcatgtctccttttttatgtactgtgttagcggtctgcttcttccagccctcctgtttgaagatggcaagttagttacgcacaataaaaaaagacctaaaatatgtaaggggtgacgccaaagtatacactttgccctttacacattttaggtcttgcctgctttatcagtaacaaacccgcgcgatttacttttcgacctcattctattagactctcgtttggattgcaactggtctattttcctcttttgtttgatagaaaatcataaaaggatttgcagactacgggcctaaagaactaaaaaatctatctgtttcttttcattctctgtattttttatagtttctgttgcatgggcataaagttgcctttttaatcacaattcagaaaatatcataatatctcatttcactaaataatagtgaacggcaggtatatgtgatgggttaaaaaggatcaccccagagtcccgctcagaagaactcgtcaagaaggcgatagaaggcgatgcgctgcgaatcgggagcggcgataccgtaaagcacgaggaagcggtcagcccattcgccgccaagctcttcagcaatatcacgggtagccaacgctatgtcctgatagcggtccgccacacccagccggccacagtcgatgaatccagaaaagcggccattttccaccatgatattcggcaagcaggcatcgccatgggtcacgacgagatcctcgccgtcgggcatccgcgccttgagcctggcgaacagttcggctggcgcgagcccctgatgctcttcgtccagatcatcctgatcgacaagaccggcttccatccgagtacgtgctcgctcgatgcgatgtttcgcttggtggtcgaatgggcaggtagccggatcaagcgtatgcagccgccgcattgcatcagccatgatggatactttctcggcaggagcaaggtgagatgacaggagatcctgccccggcacttcgcccaatagcagccagtcccttcccgcttcagtgacaacgtcgagacagctgcgcaaggaacgcccgtcgtggccagccacgatagccgcgctgcctcgtcttggagttcattcagggcaccggacaggtcggtcttgacaaaaagaaccgggcgcccctgcgctgacagccggaacacggcggcatcagagcagccgattgtctgttgtgcccagtcatagccgaatagcctctccacccaagcggccggagaacctgcgtgcaatccatcttgttcaatcatgcgaaacgatcctcatcctgtctcttgatcagatcttgatcccctgcgccatcagatccttggcggcaagaaagccatccagtttactttgcagggcttcccaaccttaccagagggcgccccagctggcaattccg